European Patent Specification EP 3 272 881 B9, published October 4, 2023. Title: Peripherical tissue sample containing cells expressing the 5HTR2C and/or ADARs as markers of the alteration of the mechanism of the 5HTR2C mRNA editing and its applications. Applicant: BIOCORTECH WEISSMANN, Dinah PUJOL, Jean-François VINCENT, Laurent CAVAREC, Laurent MANN, John. The sequence listing filed with the application follows.

SEQUENCE LISTING (51 sequences)

SEQ ID NO: 1 - DNA, 15 bp, Artificial
  Description of the artificial sequence : DNA derived from the mRNA coding for 5-HT2C receptor
atacgtaatcctatt

SEQ ID NO: 2 - DNA, 15 bp, Artificial
  Description of the artificial sequence : DNA derived from the mRNA coding for 5-HT2C receptor
  modified_base (1)..(1): n=i
ntacgtaatcctatt

SEQ ID NO: 3 - DNA, 15 bp, Artificial
  Description of the artificial sequence : DNA derived from the mRNA coding for 5-HT2C receptor
  modified_base (3)..(3): n=i
atncgtaatcctatt

SEQ ID NO: 4 - DNA, 15 bp, Artificial
  Description of the artificial sequence : DNA derived from the mRNA coding for 5-HT2C receptor
  modified_base (8)..(8): n=i
atacgtantcctatt

SEQ ID NO: 5 - DNA, 15 bp, Artificial
  Description of the artificial sequence : DNA derived from the mRNA coding for 5-HT2C receptor
  modified_base (13)..(13): n=i
atacgtaatcctntt

SEQ ID NO: 6 - DNA, 15 bp, Artificial
  Description of the artificial sequence : DNA derived from the mRNA coding for 5-HT2C receptor
  modified_base (7)..(7): n=i
atacgtnatcctatt

SEQ ID NO: 7 - DNA, 15 bp, Artificial
  Description of the artificial sequence : DNA derived from the mRNA coding for 5-HT2C receptor
  modified_base (1)..(1): n=i
  modified_base (3)..(3): n=i
ntncgtaatcctatt

SEQ ID NO: 8 - DNA, 15 bp, Artificial
  Description of the artificial sequence : DNA derived from the mRNA coding for 5-HT2C receptor
  modified_base (1)..(1): n=i
  modified_base (8)..(8): n=i
ntacgtantcctatt

SEQ ID NO: 9 - DNA, 15 bp, Artificial
  Description of the artificial sequence : DNA derived from the mRNA coding for 5-HT2C receptor
  modified_base (1)..(1): n=i
  modified_base (13)..(13): n=i
ntacgtaatcctntt

SEQ ID NO: 10 - DNA, 15 bp, Artificial
  Description of the artificial sequence : DNA derived from the mRNA coding for 5-HT2C receptor
  modified_base (1)..(1): n=i
  modified_base (7)..(7): n=i
ntacgtnatcctatt

SEQ ID NO: 11 - DNA, 15 bp, Artificial
  Description of the artificial sequence : DNA derived from the mRNA coding for 5-HT2C receptor
  modified_base (3)..(3): n=i
  modified_base (8)..(8): n=i
atncgtantcctatt

SEQ ID NO: 12 - DNA, 15 bp, Artificial
  Description of the artificial sequence : DNA derived from the mRNA coding for 5-HT2C receptor
  modified_base (3)..(3): n=i
  modified_base (13)..(13): n=i
atncgtaatcctntt

SEQ ID NO: 13 - DNA, 15 bp, Artificial
  Description of the artificial sequence : DNA derived from the mRNA coding for 5-HT2C receptor
  modified_base (3)..(3): n=i
  modified_base (7)..(7): n=i
atncgtnatcctatt

SEQ ID NO: 14 - DNA, 15 bp, Artificial
  Description of the artificial sequence : DNA derived from the mRNA coding for 5-HT2C receptor
  modified_base (8)..(8): n=i
  modified_base (13)..(13): n=i
atacgtantcctntt

SEQ ID NO: 15 - DNA, 15 bp, Artificial
  Description of the artificial sequence : DNA derived from the mRNA coding for 5-HT2C receptor
  modified_base (7)..(7): n=i
  modified_base (8)..(8): n=i
atacgtnntcctatt

SEQ ID NO: 16 - DNA, 15 bp, Artificial
  Description of the artificial sequence : DNA derived from the mRNA coding for 5-HT2C receptor
  modified_base (7)..(7): n=i
  modified_base (13)..(13): n=i
atacgtnatcctntt

SEQ ID NO: 17 - DNA, 15 bp, Artificial
  Description of the artificial sequence : DNA derived from the mRNA coding for 5-HT2C receptor
  modified_base (1)..(1): n=i
  modified_base (3)..(3): n=i
  modified_base (8)..(8): n=i
ntncgtantcctatt

SEQ ID NO: 18 - DNA, 15 bp, Artificial
  Description of the artificial sequence : DNA derived from the mRNA coding for 5-HT2C receptor
  modified_base (1)..(1): n=i
  modified_base (3)..(3): n=i
  modified_base (13)..(13): n=i
ntncgtaatcctntt

SEQ ID NO: 19 - DNA, 15 bp, Artificial
  Description of the artificial sequence : DNA derived from the mRNA coding for 5-HT2C receptor
  modified_base (1)..(1): n=i
  modified_base (3)..(3): n=i
  modified_base (7)..(7): n=i
ntncgtnatcctatt

SEQ ID NO: 20 - DNA, 15 bp, Artificial
  Description of the artificial sequence : DNA derived from the mRNA coding for 5-HT2C receptor
  modified_base (1)..(1): n=i
  modified_base (8)..(8): n=i
  modified_base (13)..(13): n=i
ntacgtantcctntt

SEQ ID NO: 21 - DNA, 15 bp, Artificial
  Description of the artificial sequence : DNA derived from the mRNA coding for 5-HT2C receptor
  modified_base (1)..(1): n=i
  modified_base (7)..(7): n=i
  modified_base (8)..(8): n=i
ntacgtnntcctatt

SEQ ID NO: 22 - DNA, 15 bp, Artificial
  Description of the artificial sequence : DNA derived from the mRNA coding for 5-HT2C receptor
  modified_base (1)..(1): n=i
  modified_base (7)..(7): n=i
  modified_base (13)..(13): n=i
ntacgtnatcctntt

SEQ ID NO: 23 - DNA, 15 bp, Artificial
  Description of the artificial sequence : DNA derived from the mRNA coding for 5-HT2C receptor
  modified_base (3)..(3): n=i
  modified_base (8)..(8): n=i
  modified_base (13)..(13): n=i
atncgtantcctntt

SEQ ID NO: 24 - DNA, 15 bp, Artificial
  Description of the artificial sequence : DNA derived from the mRNA coding for 5-HT2C receptor
  modified_base (3)..(3): n=i
  modified_base (7)..(7): n=i
  modified_base (8)..(8): n=i
atncgtnntcctatt

SEQ ID NO: 25 - DNA, 15 bp, Artificial
  Description of the artificial sequence : DNA derived from the mRNA coding for 5-HT2C receptor
  modified_base (3)..(3): n=i
  modified_base (7)..(7): n=i
  modified_base (13)..(13): n=i
atncgtnatcctntt

SEQ ID NO: 26 - DNA, 15 bp, Artificial
  Description of the artificial sequence : DNA derived from the mRNA coding for 5-HT2C receptor
  modified_base (7)..(7): n=i
  modified_base (8)..(8): n=i
  modified_base (13)..(13): n=i
atacgtnntcctntt

SEQ ID NO: 27 - DNA, 15 bp, Artificial
  Description of the artificial sequence : DNA derived from the mRNA coding for 5-HT2C receptor
  modified_base (1)..(1): n=i
  modified_base (3)..(3): n=i
  modified_base (8)..(8): n=i
  modified_base (13)..(13): n=i
ntncgtantcctntt

SEQ ID NO: 28 - DNA, 15 bp, Artificial
  Description of the artificial sequence : DNA derived from the mRNA coding for 5-HT2C receptor
  modified_base (1)..(1): n=i
  modified_base (3)..(3): n=i
  modified_base (7)..(7): n=i
  modified_base (8)..(8): n=i
ntncgtnntcctatt

SEQ ID NO: 29 - DNA, 15 bp, Artificial
  Description of the artificial sequence : DNA derived from the mRNA coding for 5-HT2C receptor
  modified_base (1)..(1): n=i
  modified_base (3)..(3): n=i
  modified_base (7)..(7): n=i
  modified_base (13)..(13): n=i
ntncgtnatcctntt

SEQ ID NO: 30 - DNA, 15 bp, Artificial
  Description of the artificial sequence : DNA derived from the mRNA coding for 5-HT2C receptor
  modified_base (1)..(1): n=i
  modified_base (7)..(7): n=i
  modified_base (8)..(8): n=i
  modified_base (13)..(13): n=i
ntacgtnntcctntt

SEQ ID NO: 31 - DNA, 15 bp, Artificial
  Description of the artificial sequence : DNA derived from the mRNA coding for 5-HT2C receptor
  modified_base (3)..(3): n=i
  modified_base (7)..(7): n=i
  modified_base (8)..(8): n=i
  modified_base (13)..(13): n=i
atncgtnntcctntt

SEQ ID NO: 32 - DNA, 15 bp, Artificial
  Description of the artificial sequence : DNA derived from the mRNA coding for 5-HT2C receptor
  modified_base (1)..(1): n=i
  modified_base (3)..(3): n=i
  modified_base (7)..(7): n=i
  modified_base (8)..(8): n=i
  modified_base (13)..(13): n=i
ntncgtnntcctntt

SEQ ID NO: 33 - RNA, 15 nt, Artificial
  Description of the artificial sequence : sequence derived from the cDNA coding for 5-HT2C receptor
auacguaauccuauu

SEQ ID NO: 34 - DNA, 21 bp, Artificial
  Description of the artificial sequence : sequence derived from the cDNA coding for 5-HT2C receptor
ttcgtccctcagtccaatcac

SEQ ID NO: 35 - DNA, 24 bp, Artificial
  Description of the artificial sequence : sequence derived from the cDNA coding for 5-HT2C receptor
tgtccctagccattgctgatatgc

SEQ ID NO: 36 - DNA, 24 bp, Artificial
  Description of the artificial sequence : sequence derived from the cDNA coding for 5-HT2C receptor
gcaatcttcatgatggccttagtc

SEQ ID NO: 37 - DNA, 26 bp, Artificial
  Description of the artificial sequence : sequence derived from the cDNA coding for 5-HT2C receptor
atgtgctattttcaacagcgtccatc

SEQ ID NO: 38 - DNA, 21 bp, Artificial
  Description of the artificial sequence : sequence derived from the cDNA coding for 5-HT2C receptor
gcaatcttcatgatggcctta

SEQ ID NO: 39 - DNA, 18 bp, Artificial
  Description of the artificial sequence : sequence derived from the cDNA coding for 5-HT2C receptor
tttgtgccccgtctggat

SEQ ID NO: 40 - DNA, 18 bp, Artificial
  Description of the artificial sequence : sequence derived from the cDNA coding for 5-HT2C receptor
gccttagtccgcgaattg

SEQ ID NO: 41 - DNA, 22 bp, Artificial
  Description of the artificial sequence : sequence derived from the cDNA coding for human ADAR1 150 isoform
gcctcgcgggcgcaatgaatcc

SEQ ID NO: 42 - DNA, 22 bp, Artificial
  Description of the artificial sequence : sequence derived from the cDNA coding for human ADAR1 150 isoform
cttgcccttctttgccagggag

SEQ ID NO: 43 - DNA, 24 bp, Artificial
  Description of the artificial sequence : sequence derived from the cDNA coding for human ADAR1 110 isoform
cgagccatcatggagatgccctcc

SEQ ID NO: 44 - DNA, 24 bp, Artificial
  Description of the artificial sequence : sequence derived from the cDNA coding for human ADAR1 110 isoform
catagctgcatcctgcttggccac

SEQ ID NO: 45 - DNA, 23 bp, Artificial
  Description of the artificial sequence : sequence derived from the cDNA coding for human ADAR2
gctgcgcagtctgccctggccgc

SEQ ID NO: 46 - DNA, 23 bp, Artificial
  Description of the artificial sequence : sequence derived from the cDNA coding for human ADAR2
gtcatgacgactccagccagcac

SEQ ID NO: 47 - DNA, 22 bp, Artificial
  Description of the artificial sequence : sequence derived from the cDNA coding for murine ADAR1 150 isoform
gtctcaagggttcaggggaccc

SEQ ID NO: 48 - DNA, 24 bp, Artificial
  Description of the artificial sequence : sequence derived from the cDNA coding for murine ADAR1 150 isoform
ctcctctagggaattcctggatac

SEQ ID NO: 49 - DNA, 23 bp, Artificial
  Description of the artificial sequence : sequence derived from the cDNA coding for murine ADAR1 110 isoform
tcacgagtgggcagcgtccgagg

SEQ ID NO: 50 - DNA, 23 bp, Artificial
  Description of the artificial sequence : sequence derived from the cDNA coding for murine ADAR2
gctgcacagtctgccttggctac

SEQ ID NO: 51 - DNA, 24 bp, Artificial
  Description of the artificial sequence : sequence derived from the cDNA coding for murine ADAR2
gcataaagaaacctgagcagggac